European Patent Application EP 4 617 281 A1, published September 17, 2025. Title: SITE-SPECIFIC PEGYLATED HETEROMERIC PROTEIN OR POLYPEPTIDE, AND PREPARATION METHOD THEREFOR AND USE THEREOF. Applicant: KANGLITAI BIOMEDICAL (QINGDAO) CO.,LTD. Application CN PCT/CN2023/131105, filed November 10, 2023. The sequence listing filed with the application follows.

SEQUENCE LISTING (70 sequences)

SEQ ID NO: 1 - protein, 197 aa, Homo sapiens
RNLPVATPDPGMFPCLHHSQNLLRAVSNMLQKARQTLEFYPCTSEEIDHEDITKDKTSTVEACLPLELTKNESCLNSRETSFITNGSCLASRKTSFMMALCLSSIYEDLKMYQVEFKTMNAKLLMDPKRQIFLDQNMLAVIDELMQALNFNSETVPQKSSLEEPDFYKTKIKLCILLHAFRIRAVTIDRVMSYLNAS

SEQ ID NO: 2 - protein, 306 aa, Homo sapiens
IWELKKDVYVVELDWYPDAPGEMVVLTCDTPEEDGITWTLDQSSEVLGSGKTLTIQVKEFGDAGQYTCHKGGEVLSHSLLLLHKKEDGIWSTDILKDQKEPKNKTFLRCEAKNYSGRFTCWWLTTISTDLTFSVKSSRGSSDPQGVTCGAATLSAERVRGDNKEYEYSVECQEDSACPAAEESLPIEVMVDAVHKLKYENYTSSFFIRDIIKPDPPKNLQLKPLKNSRQVEVSWEYPDTWSTPHSYFSLTFCVQVQGKSKREKKDRVFTDKTSATVICRKNASISVRAQDRYYSSSWSEWASVPCS

SEQ ID NO: 3 - protein, 197 aa, synthetic construct
PNLPVATPDPGMFPCLHHSQNLLRAVSNMLQKARQTLEFYPCTSEEIDHEDITKDKTSTVEACLPLELTKNESCLNSRETSFITNGSCLASRKTSFMMALCLSSIYEDLKMYQVEFKTMNAKLLMDPKRQIFLDQNMLAVIDELMQALNFNSETVPQKSSLEEPDFYKTKIKLCILLHAFRIRAVTIDRVMSYLNAS

SEQ ID NO: 4 - protein, 197 aa, synthetic construct
QNLPVATPDPGMFPCLHHSQNLLRAVSNMLQKARQTLEFYPCTSEEIDHEDITKDKTSTVEACLPLELTKNESCLNSRETSFITNGSCLASRKTSFMMALCLSSIYEDLKMYQVEFKTMNAKLLMDPKRQIFLDQNMLAVIDELMQALNFNSETVPQKSSLEEPDFYKTKIKLCILLHAFRIRAVTIDRVMSYLNAS

SEQ ID NO: 5 - protein, 197 aa, synthetic construct
NNLPVATPDPGMFPCLHHSQNLLRAVSNMLQKARQTLEFYPCTSEEIDHEDITKDKTSTVEACLPLELTKNESCLNSRETSFITNGSCLASRKTSFMMALCLSSIYEDLKMYQVEFKTMNAKLLMDPKRQIFLDQNMLAVIDELMQALNFNSETVPQKSSLEEPDFYKTKIKLCILLHAFRIRAVTIDRVMSYLNAS

SEQ ID NO: 6 - protein, 306 aa, synthetic construct
PWELKKDVYVVELDWYPDAPGEMVVLTCDTPEEDGITWTLDQSSEVLGSGKTLTIQVKEFGDAGQYTCHKGGEVLSHSLLLLHKKEDGIWSTDILKDQKEPKNKTFLRCEAKNYSGRFTCWWLTTISTDLTFSVKSSRGSSDPQGVTCGAATLSAERVRGDNKEYEYSVECQEDSACPAAEESLPIEVMVDAVHKLKYENYTSSFFIRDIIKPDPPKNLQLKPLKNSRQVEVSWEYPDTWSTPHSYFSLTFCVQVQGKSKREKKDRVFTDKTSATVICRKNASISVRAQDRYYSSSWSEWASVPCS

SEQ ID NO: 7 - protein, 306 aa, synthetic construct
QWELKKDVYVVELDWYPDAPGEMVVLTCDTPEEDGITWTLDQSSEVLGSGKTLTIQVKEFGDAGQYTCHKGGEVLSHSLLLLHKKEDGIWSTDILKDQKEPKNKTFLRCEAKNYSGRFTCWWLTTISTDLTFSVKSSRGSSDPQGVTCGAATLSAERVRGDNKEYEYSVECQEDSACPAAEESLPIEVMVDAVHKLKYENYTSSFFIRDIIKPDPPKNLQLKPLKNSRQVEVSWEYPDTWSTPHSYFSLTFCVQVQGKSKREKKDRVFTDKTSATVICRKNASISVRAQDRYYSSSWSEWASVPCS

SEQ ID NO: 8 - protein, 306 aa, synthetic construct
NWELKKDVYVVELDWYPDAPGEMVVLTCDTPEEDGITWTLDQSSEVLGSGKTLTIQVKEFGDAGQYTCHKGGEVLSHSLLLLHKKEDGIWSTDILKDQKEPKNKTFLRCEAKNYSGRFTCWWLTTISTDLTFSVKSSRGSSDPQGVTCGAATLSAERVRGDNKEYEYSVECQEDSACPAAEESLPIEVMVDAVHKLKYENYTSSFFIRDIIKPDPPKNLQLKPLKNSRQVEVSWEYPDTWSTPHSYFSLTFCVQVQGKSKREKKDRVFTDKTSATVICRKNASISVRAQDRYYSSSWSEWASVPCS

SEQ ID NO: 9 - protein, 193 aa, Mus musculus
RVIPVSGPARCLSQSRNLLKTTDDMVKTAREKLKHYSCTAEDIDHEDITRDQTSTLKTCLPLELHKNESCLATRETSSTTRGSCLPPQKTSLMMTLCLGSIYEDLKMYQTEFQAINAALQNHNHQQIILDKGMLVAIDELMQSLNHNGETLRQKPPVGEADPYRVKMKLCILLHAFSTRVVTINRVMGYLSSA

SEQ ID NO: 10 - protein, 313 aa, Mus musculus
MWELEKDVYVVEVDWTPDAPGETVNLTCDTPEEDDITWTSDQRHGVIGSGKTLTITVKEFLDAGQYTCHKGGETLSHSHLLLHKKENGIWSTEILKNFKNKTFLKCEAPNYSGRFTCSWLVQRNMDLKFNIKSSSSSPDSRAVTCGMASLSAEKVTLDQRDYEKYSVSCQEDVTCPTAEETLPIELALEARQQNKYENYSTSFFIRDIIKPDPPKNLQMKPLKNSQVEVSWEYPDSWSTPHSYFSLKFFVRIQRKKEKMKETEEGCNQKGAFLVEKTSTEVQCKGGNVCVQAQDRYYNSSCSKWACVPCRVRS

SEQ ID NO: 11 - protein, 192 aa, synthetic construct
PVIPVSGPARCLSQSRNLLKTTDDMVKTAREKLKHYSCTAEDIDHEDITRDQTSTLKTCLPLELHKNESCLATRETSSTTRGSCLPPQKTSLMMTLCLGSIYEDLKMYQTEFQAINAALQNHNHQQIILDKGMLVAIDELMQSLNHNGETLRQKPPVGEADPYRVKMKLCILLHAFSTRVVTINRVMGYLSS

SEQ ID NO: 12 - protein, 192 aa, synthetic construct
QVIPVSGPARCLSQSRNLLKTTDDMVKTAREKLKHYSCTAEDIDHEDITRDQTSTLKTCLPLELHKNESCLATRETSSTTRGSCLPPQKTSLMMTLCLGSIYEDLKMYQTEFQAINAALQNHNHQQIILDKGMLVAIDELMQSLNHNGETLRQKPPVGEADPYRVKMKLCILLHAFSTRVVTINRVMGYLSS

SEQ ID NO: 13 - protein, 192 aa, synthetic construct
NVIPVSGPARCLSQSRNLLKTTDDMVKTAREKLKHYSCTAEDIDHEDITRDQTSTLKTCLPLELHKNESCLATRETSSTTRGSCLPPQKTSLMMTLCLGSIYEDLKMYQTEFQAINAALQNHNHQQIILDKGMLVAIDELMQSLNHNGETLRQKPPVGEADPYRVKMKLCILLHAFSTRVVTINRVMGYLSS

SEQ ID NO: 14 - protein, 313 aa, synthetic construct
PWELEKDVYVVEVDWTPDAPGETVNLTCDTPEEDDITWTSDQRHGVIGSGKTLTITVKEFLDAGQYTCHKGGETLSHSHLLLHKKENGIWSTEILKNFKNKTFLKCEAPNYSGRFTCSWLVQRNMDLKFNIKSSSSSPDSRAVTCGMASLSAEKVTLDQRDYEKYSVSCQEDVTCPTAEETLPIELALEARQQNKYENYSTSFFIRDIIKPDPPKNLQMKPLKNSQVEVSWEYPDSWSTPHSYFSLKFFVRIQRKKEKMKETEEGCNQKGAFLVEKTSTEVQCKGGNVCVQAQDRYYNSSCSKWACVPCRVRS

SEQ ID NO: 15 - protein, 313 aa, synthetic construct
QWELEKDVYVVEVDWTPDAPGETVNLTCDTPEEDDITWTSDQRHGVIGSGKTLTITVKEFLDAGQYTCHKGGETLSHSHLLLHKKENGIWSTEILKNFKNKTFLKCEAPNYSGRFTCSWLVQRNMDLKFNIKSSSSSPDSRAVTCGMASLSAEKVTLDQRDYEKYSVSCQEDVTCPTAEETLPIELALEARQQNKYENYSTSFFIRDIIKPDPPKNLQMKPLKNSQVEVSWEYPDSWSTPHSYFSLKFFVRIQRKKEKMKETEEGCNQKGAFLVEKTSTEVQCKGGNVCVQAQDRYYNSSCSKWACVPCRVRS

SEQ ID NO: 16 - protein, 313 aa, synthetic construct
NWELEKDVYVVEVDWTPDAPGETVNLTCDTPEEDDITWTSDQRHGVIGSGKTLTITVKEFLDAGQYTCHKGGETLSHSHLLLHKKENGIWSTEILKNFKNKTFLKCEAPNYSGRFTCSWLVQRNMDLKFNIKSSSSSPDSRAVTCGMASLSAEKVTLDQRDYEKYSVSCQEDVTCPTAEETLPIELALEARQQNKYENYSTSFFIRDIIKPDPPKNLQMKPLKNSQVEVSWEYPDSWSTPHSYFSLKFFVRIQRKKEKMKETEEGCNQKGAFLVEKTSTEVQCKGGNVCVQAQDRYYNSSCSKWACVPCRVRS

SEQ ID NO: 17 - protein, 92 aa, Homo sapiens
APDVQDCPECTLQENPFFSQPGAPILQCMGCCFSRAYPTPLRSKKTMLVQKNVTSESTCCVAKSYNRVTVMGGFKVENHTACHCSTCYYHKS

SEQ ID NO: 18 - protein, 121 aa, Homo sapiens
SREPLRPWCHPINAILAVEKEGCPVCITVNTTICAGYCPTMMRVLQAVLPPLPQVVCTYRDVRFESIRLPGCPRGVDPVVSFPVALSCRCGPCRRSTSDCGGPKDHPLTCDHPQLSGLLFL

SEQ ID NO: 19 - protein, 118 aa, Homo sapiens
FCIPTEYTMHIERRECAYCLTINTTICAGYCMTRDINGKLFLPKYALSQDVCTYRDFIYRTVEIPGCPLHVAPYFSYPVALSCKCGKCNTDYSDCIHEAIKTNYCTKPQKSYLVGFSV

SEQ ID NO: 20 - protein, 111 aa, Homo sapiens
NSCELTNITIAIEKEECRFCISINTTWCAGYCYTRDLVYKDPARPKIQKTCTFKELVYETVRVPGCAHHADSLYTYPVATQCHCGKCDSDSTDCTVRGLGPSYCSFGEMKE

SEQ ID NO: 21 - protein, 145 aa, Homo sapiens
SKEPLRPRCRPINATLAVEKEGCPVCITVNTTICAGYCPTMTRVLQGVLPALPQVVCNYRDVRFESIRLPGCPRGVNPVVSYAVALSCQCALCRRSTTDCGGPKDHPLTCDDPRFQASSSSKAPPPSLPSPSRLPGPSDTPILPQ

SEQ ID NO: 22 - protein, 145 aa, Homo sapiens
SKEPLRPRCRPINATLAVEKEGCPVCITVNTTICAGYCPTMTRVLQGVLPALPQVVCNYRDVRFESIRLPGCPRGVNPVVSYAVALSCQCALCRRSTTDCGGPKDHPLTCDDPRFQDSSSSKAPPPSLPSPSRLPGPSDTPILPQ

SEQ ID NO: 23 - protein, 145 aa, Homo sapiens; identical to SEQ ID NO: 22

SEQ ID NO: 24 - protein, 145 aa, Homo sapiens
SREMLRPRCRPINATLAVEKEGCPVCITVNTTICAGYCPTMTRVLQGVLPALPQVVCNYRDVRFESIRLPGCPRGVNPVVSYAVALSCQCALCRRSTTDCGGPKDHPLTCDDPRFQASSSSKAPPPSLPSPSRLPGPSDTPILPQ

SEQ ID NO: 25 - protein, 145 aa, Homo sapiens; identical to SEQ ID NO: 24

SEQ ID NO: 26 - protein, 92 aa, synthetic construct
PPDVQDCPECTLQENPFFSQPGAPILQCMGCCFSRAYPTPLRSKKTMLVQKNVTSESTCCVAKSYNRVTVMGGFKVENHTACHCSTCYYHKS

SEQ ID NO: 27 - protein, 92 aa, synthetic construct
QPDVQDCPECTLQENPFFSQPGAPILQCMGCCFSRAYPTPLRSKKTMLVQKNVTSESTCCVAKSYNRVTVMGGFKVENHTACHCSTCYYHKS

SEQ ID NO: 28 - protein, 92 aa, synthetic construct
NPDVQDCPECTLQENPFFSQPGAPILQCMGCCFSRAYPTPLRSKKTMLVQKNVTSESTCCVAKSYNRVTVMGGFKVENHTACHCSTCYYHKS

SEQ ID NO: 29 - protein, 96 aa, Mus musculus
LPDGDFIIQGCPECKLKENKYFSKLGAPIYQCMGCCFSRAYPTPARSKKTMLVPKNITSEATCCVAKAFTKATVMGNARVENHTECHCSTCYYHKS

SEQ ID NO: 30 - protein, 121 aa, Mus musculus
SRGPLRPLCRPVNATLAAENEFCPVCITFTTSICAGYCPSMVRVLPAALPPVPQPVCTYRELAFASVRLPGCPPGVDPIVSFPVALSCRCGPCRLSSSDCGGPRTQPMACDLPHLPGLLLL

SEQ ID NO: 31 - protein, 118 aa, Mus musculus
FCIPTEYTMYVDRRECAYCLTINTTICAGYCMTRDINGKLFLPKYALSQDVCTYRDFIYRTVEIPGCPHHVTPYFSFPVAVSCKCGKCNTDNSDCIHEAVRTNYCTKPQSFYLGGFSV

SEQ ID NO: 32 - protein, 109 aa, Mus musculus
CELTNITISVEKEECRFCISINTTWCAGYCYTRDLVYKDPARPNTQKVCTFKELVYETVRLPGCARHSDSLYTYPVATECHCGKCDSDSTDCTVRGLGPSYCSFSEMKE

SEQ ID NO: 33 - protein, 96 aa, synthetic construct
PPDGDFIIQGCPECKLKENKYFSKLGAPIYQCMGCCFSRAYPTPARSKKTMLVPKNITSEATCCVAKAFTKATVMGNARVENHTECHCSTCYYHKS

SEQ ID NO: 34 - protein, 96 aa, synthetic construct
QPDGDFIIQGCPECKLKENKYFSKLGAPIYQCMGCCFSRAYPTPARSKKTMLVPKNITSEATCCVAKAFTKATVMGNARVENHTECHCSTCYYHKS

SEQ ID NO: 35 - protein, 96 aa, synthetic construct
NPDGDFIIQGCPECKLKENKYFSKLGAPIYQCMGCCFSRAYPTPARSKKTMLVPKNITSEATCCVAKAFTKATVMGNARVENHTECHCSTCYYHKS

SEQ ID NO: 36 - DNA, 591 bp, Homo sapiens
  source 1..591: mol_type = other DNA
cgcaacctgccggtggcgaccccggatccgggcatgtttccgtgcctgcatcatagccagaacctgctgcgcgcggtgagcaacatgctgcagaaagcgcgccagaccctggaattttatccgtgcaccagcgaagaaattgatcatgaagatattaccaaagataaaaccagcaccgtggaagcgtgcctgccgctggaactgaccaaaaacgaaagctgcctgaacagccgcgaaaccagctttattaccaacggcagctgcctggcgagccgcaaaaccagctttatgatggcgctgtgcctgagcagcatttatgaagatctgaaaatgtatcaggtggaatttaaaaccatgaacgcgaaactgctgatggatccgaaacgccagatttttctggatcagaacatgctggcggtgattgatgaactgatgcaggcgctgaactttaacagcgaaaccgtgccgcagaaaagcagcctggaagaaccggatttttataaaaccaaaattaaactgtgcattctgctgcatgcgtttcgcattcgcgcggtgaccattgatcgcgtgatgagctatctgaacgcgagc

SEQ ID NO: 37 - DNA, 918 bp, Homo sapiens
  source 1..918: mol_type = genomic DNA
atttgggaactgaaaaaagatgtgtatgtggtggaactggattggtatccggatgcgccgggcgaaatggtggtgctgacctgcgataccccggaagaagatggcattacctggaccctggatcagagcagcgaagtgctgggcagcggcaaaaccctgaccattcaggtgaaagaatttggcgatgcgggccagtatacctgccataaaggcggcgaagtgctgagccatagcctgctgctgctgcataaaaaagaagatggcatttggagcaccgatattctgaaagatcagaaagaaccgaaaaacaaaacctttctgcgctgcgaagcgaaaaactatagcggccgctttacctgctggtggctgaccaccattagcaccgatctgacctttagcgtgaaaagcagccgcggcagcagcgatccgcagggcgtgacctgcggcgcggcgaccctgagcgcggaacgcgtgcgcggcgataacaaagaatatgaatatagcgtggaatgccaggaagatagcgcgtgcccggcggcggaagaaagcctgccgattgaagtgatggtggatgcggtgcataaactgaaatatgaaaactataccagcagcttttttattcgcgatattattaaaccggatccgccgaaaaacctgcagctgaaaccgctgaaaaacagccgccaggtggaagtgagctgggaatatccggatacctggagcaccccgcatagctattttagcctgaccttttgcgtgcaggtgcagggcaaaagcaaacgcgaaaaaaaagatcgcgtgtttaccgataaaaccagcgcgaccgtgatttgccgcaaaaacgcgagcattagcgtgcgcgcgcaggatcgctattatagcagcagctggagcgaatgggcgagcgtgccgtgcagc

SEQ ID NO: 38 - DNA, 591 bp, synthetic construct
  source 1..591: mol_type = other DNA
ccgaacctgccggtggcgaccccggatccgggcatgtttccgtgcctgcatcatagccagaacctgctgcgcgcggtgagcaacatgctgcagaaagcgcgccagaccctggaattttatccgtgcaccagcgaagaaattgatcatgaagatattaccaaagataaaaccagcaccgtggaagcgtgcctgccgctggaactgaccaaaaacgaaagctgcctgaacagccgcgaaaccagctttattaccaacggcagctgcctggcgagccgcaaaaccagctttatgatggcgctgtgcctgagcagcatttatgaagatctgaaaatgtatcaggtggaatttaaaaccatgaacgcgaaactgctgatggatccgaaacgccagatttttctggatcagaacatgctggcggtgattgatgaactgatgcaggcgctgaactttaacagcgaaaccgtgccgcagaaaagcagcctggaagaaccggatttttataaaaccaaaattaaactgtgcattctgctgcatgcgtttcgcattcgcgcggtgaccattgatcgcgtgatgagctatctgaacgcgagc

SEQ ID NO: 39 - DNA, 591 bp, synthetic construct
  source 1..591: mol_type = other DNA
cagaacctgccggtggcgaccccggatccgggcatgtttccgtgcctgcatcatagccagaacctgctgcgcgcggtgagcaacatgctgcagaaagcgcgccagaccctggaattttatccgtgcaccagcgaagaaattgatcatgaagatattaccaaagataaaaccagcaccgtggaagcgtgcctgccgctggaactgaccaaaaacgaaagctgcctgaacagccgcgaaaccagctttattaccaacggcagctgcctggcgagccgcaaaaccagctttatgatggcgctgtgcctgagcagcatttatgaagatctgaaaatgtatcaggtggaatttaaaaccatgaacgcgaaactgctgatggatccgaaacgccagatttttctggatcagaacatgctggcggtgattgatgaactgatgcaggcgctgaactttaacagcgaaaccgtgccgcagaaaagcagcctggaagaaccggatttttataaaaccaaaattaaactgtgcattctgctgcatgcgtttcgcattcgcgcggtgaccattgatcgcgtgatgagctatctgaacgcgagc

SEQ ID NO: 40 - DNA, 591 bp, synthetic construct
  source 1..591: mol_type = other DNA
aacaacctgccggtggcgaccccggatccgggcatgtttccgtgcctgcatcatagccagaacctgctgcgcgcggtgagcaacatgctgcagaaagcgcgccagaccctggaattttatccgtgcaccagcgaagaaattgatcatgaagatattaccaaagataaaaccagcaccgtggaagcgtgcctgccgctggaactgaccaaaaacgaaagctgcctgaacagccgcgaaaccagctttattaccaacggcagctgcctggcgagccgcaaaaccagctttatgatggcgctgtgcctgagcagcatttatgaagatctgaaaatgtatcaggtggaatttaaaaccatgaacgcgaaactgctgatggatccgaaacgccagatttttctggatcagaacatgctggcggtgattgatgaactgatgcaggcgctgaactttaacagcgaaaccgtgccgcagaaaagcagcctggaagaaccggatttttataaaaccaaaattaaactgtgcattctgctgcatgcgtttcgcattcgcgcggtgaccattgatcgcgtgatgagctatctgaacgcgagc

SEQ ID NO: 41 - DNA, 918 bp, synthetic construct
  source 1..918: mol_type = other DNA
ccgtgggaactgaaaaaagatgtgtatgtggtggaactggattggtatccggatgcgccgggcgaaatggtggtgctgacctgcgataccccggaagaagatggcattacctggaccctggatcagagcagcgaagtgctgggcagcggcaaaaccctgaccattcaggtgaaagaatttggcgatgcgggccagtatacctgccataaaggcggcgaagtgctgagccatagcctgctgctgctgcataaaaaagaagatggcatttggagcaccgatattctgaaagatcagaaagaaccgaaaaacaaaacctttctgcgctgcgaagcgaaaaactatagcggccgctttacctgctggtggctgaccaccattagcaccgatctgacctttagcgtgaaaagcagccgcggcagcagcgatccgcagggcgtgacctgcggcgcggcgaccctgagcgcggaacgcgtgcgcggcgataacaaagaatatgaatatagcgtggaatgccaggaagatagcgcgtgcccggcggcggaagaaagcctgccgattgaagtgatggtggatgcggtgcataaactgaaatatgaaaactataccagcagcttttttattcgcgatattattaaaccggatccgccgaaaaacctgcagctgaaaccgctgaaaaacagccgccaggtggaagtgagctgggaatatccggatacctggagcaccccgcatagctattttagcctgaccttttgcgtgcaggtgcagggcaaaagcaaacgcgaaaaaaaagatcgcgtgtttaccgataaaaccagcgcgaccgtgatttgccgcaaaaacgcgagcattagcgtgcgcgcgcaggatcgctattatagcagcagctggagcgaatgggcgagcgtgccgtgcagc

SEQ ID NO: 42 - DNA, 918 bp, synthetic construct
  source 1..918: mol_type = other DNA
cagtgggaactgaaaaaagatgtgtatgtggtggaactggattggtatccggatgcgccgggcgaaatggtggtgctgacctgcgataccccggaagaagatggcattacctggaccctggatcagagcagcgaagtgctgggcagcggcaaaaccctgaccattcaggtgaaagaatttggcgatgcgggccagtatacctgccataaaggcggcgaagtgctgagccatagcctgctgctgctgcataaaaaagaagatggcatttggagcaccgatattctgaaagatcagaaagaaccgaaaaacaaaacctttctgcgctgcgaagcgaaaaactatagcggccgctttacctgctggtggctgaccaccattagcaccgatctgacctttagcgtgaaaagcagccgcggcagcagcgatccgcagggcgtgacctgcggcgcggcgaccctgagcgcggaacgcgtgcgcggcgataacaaagaatatgaatatagcgtggaatgccaggaagatagcgcgtgcccggcggcggaagaaagcctgccgattgaagtgatggtggatgcggtgcataaactgaaatatgaaaactataccagcagcttttttattcgcgatattattaaaccggatccgccgaaaaacctgcagctgaaaccgctgaaaaacagccgccaggtggaagtgagctgggaatatccggatacctggagcaccccgcatagctattttagcctgaccttttgcgtgcaggtgcagggcaaaagcaaacgcgaaaaaaaagatcgcgtgtttaccgataaaaccagcgcgaccgtgatttgccgcaaaaacgcgagcattagcgtgcgcgcgcaggatcgctattatagcagcagctggagcgaatgggcgagcgtgccgtgcagc

SEQ ID NO: 43 - DNA, 918 bp, synthetic construct
  source 1..918: mol_type = other DNA
aactgggaactgaaaaaagatgtgtatgtggtggaactggattggtatccggatgcgccgggcgaaatggtggtgctgacctgcgataccccggaagaagatggcattacctggaccctggatcagagcagcgaagtgctgggcagcggcaaaaccctgaccattcaggtgaaagaatttggcgatgcgggccagtatacctgccataaaggcggcgaagtgctgagccatagcctgctgctgctgcataaaaaagaagatggcatttggagcaccgatattctgaaagatcagaaagaaccgaaaaacaaaacctttctgcgctgcgaagcgaaaaactatagcggccgctttacctgctggtggctgaccaccattagcaccgatctgacctttagcgtgaaaagcagccgcggcagcagcgatccgcagggcgtgacctgcggcgcggcgaccctgagcgcggaacgcgtgcgcggcgataacaaagaatatgaatatagcgtggaatgccaggaagatagcgcgtgcccggcggcggaagaaagcctgccgattgaagtgatggtggatgcggtgcataaactgaaatatgaaaactataccagcagcttttttattcgcgatattattaaaccggatccgccgaaaaacctgcagctgaaaccgctgaaaaacagccgccaggtggaagtgagctgggaatatccggatacctggagcaccccgcatagctattttagcctgaccttttgcgtgcaggtgcagggcaaaagcaaacgcgaaaaaaaagatcgcgtgtttaccgataaaaccagcgcgaccgtgatttgccgcaaaaacgcgagcattagcgtgcgcgcgcaggatcgctattatagcagcagctggagcgaatgggcgagcgtgccgtgcagc

SEQ ID NO: 44 - DNA, 579 bp, Mus musculus
  source 1..579: mol_type = genomic DNA
cgcgtgattccggtgagcggcccggcgcgctgcctgagccagagccgcaacctgctgaaaaccaccgatgatatggtgaaaaccgcgcgcgaaaaactgaaacattatagctgcaccgcggaagatattgatcatgaagatattacccgcgatcagaccagcaccctgaaaacctgcctgccgctggaactgcataaaaacgaaagctgcctggcgacccgcgaaaccagcagcaccacccgcggcagctgcctgccgccgcagaaaaccagcctgatgatgaccctgtgcctgggcagcatttatgaagatctgaaaatgtatcagaccgaatttcaggcgattaacgcggcgctgcagaaccataaccatcagcagattattctggataaaggcatgctggtggcgattgatgaactgatgcagagcctgaaccataacggcgaaaccctgcgccagaaaccgccggtgggcgaagcggatccgtatcgcgtgaaaatgaaactgtgcattctgctgcatgcgtttagcacccgcgtggtgaccattaaccgcgtgatgggctatctgagcagcgcg

SEQ ID NO: 45 - DNA, 939 bp, Mus musculus
  source 1..939: mol_type = genomic DNA
atgtgggaactggaaaaagatgtgtatgtggtggaagtggattggaccccggatgcgccgggcgaaaccgtgaacctgacctgcgataccccggaagaagatgatattacctggaccagcgatcagcgccatggcgtgattggcagcggcaaaaccctgaccattaccgtgaaagaatttctggatgcgggccagtatacctgccataaaggcggcgaaaccctgagccatagccatctgctgctgcataaaaaagaaaacggcatttggagcaccgaaattctgaaaaactttaaaaacaaaacctttctgaaatgcgaagcgccgaactatagcggccgctttacctgcagctggctggtgcagcgcaacatggatctgaaatttaacattaaaagcagcagcagcagcccggatagccgcgcggtgacctgcggcatggcgagcctgagcgcggaaaaagtgaccctggatcagcgcgattatgaaaaatatagcgtgagctgccaggaagatgtgacctgcccgaccgcggaagaaaccctgccgattgaactggcgctggaagcgcgccagcagaacaaatatgaaaactatagcaccagcttttttattcgcgatattattaaaccggatccgccgaaaaacctgcagatgaaaccgctgaaaaacagccaggtggaagtgagctgggaatatccggatagctggagcaccccgcatagctattttagcctgaaattttttgtgcgcattcagcgcaaaaaagaaaaaatgaaagaaaccgaagaaggctgcaaccagaaaggcgcgtttctggtggaaaaaaccagcaccgaagtgcagtgcaaaggcggcaacgtgtgcgtgcaggcgcaggatcgctattataacagcagctgcagcaaatgggcgtgcgtgccgtgccgcgtgcgcagc

SEQ ID NO: 46 - DNA, 576 bp, synthetic construct
  source 1..576: mol_type = other DNA
ccggtgattccggtgagcggcccggcgcgctgcctgagccagagccgcaacctgctgaaaaccaccgatgatatggtgaaaaccgcgcgcgaaaaactgaaacattatagctgcaccgcggaagatattgatcatgaagatattacccgcgatcagaccagcaccctgaaaacctgcctgccgctggaactgcataaaaacgaaagctgcctggcgacccgcgaaaccagcagcaccacccgcggcagctgcctgccgccgcagaaaaccagcctgatgatgaccctgtgcctgggcagcatttatgaagatctgaaaatgtatcagaccgaatttcaggcgattaacgcggcgctgcagaaccataaccatcagcagattattctggataaaggcatgctggtggcgattgatgaactgatgcagagcctgaaccataacggcgaaaccctgcgccagaaaccgccggtgggcgaagcggatccgtatcgcgtgaaaatgaaactgtgcattctgctgcatgcgtttagcacccgcgtggtgaccattaaccgcgtgatgggctatctgagcagc

SEQ ID NO: 47 - DNA, 576 bp, synthetic construct
  source 1..576: mol_type = other DNA
caggtgattccggtgagcggcccggcgcgctgcctgagccagagccgcaacctgctgaaaaccaccgatgatatggtgaaaaccgcgcgcgaaaaactgaaacattatagctgcaccgcggaagatattgatcatgaagatattacccgcgatcagaccagcaccctgaaaacctgcctgccgctggaactgcataaaaacgaaagctgcctggcgacccgcgaaaccagcagcaccacccgcggcagctgcctgccgccgcagaaaaccagcctgatgatgaccctgtgcctgggcagcatttatgaagatctgaaaatgtatcagaccgaatttcaggcgattaacgcggcgctgcagaaccataaccatcagcagattattctggataaaggcatgctggtggcgattgatgaactgatgcagagcctgaaccataacggcgaaaccctgcgccagaaaccgccggtgggcgaagcggatccgtatcgcgtgaaaatgaaactgtgcattctgctgcatgcgtttagcacccgcgtggtgaccattaaccgcgtgatgggctatctgagcagc

SEQ ID NO: 48 - DNA, 576 bp, synthetic construct
  source 1..576: mol_type = other DNA
aacgtgattccggtgagcggcccggcgcgctgcctgagccagagccgcaacctgctgaaaaccaccgatgatatggtgaaaaccgcgcgcgaaaaactgaaacattatagctgcaccgcggaagatattgatcatgaagatattacccgcgatcagaccagcaccctgaaaacctgcctgccgctggaactgcataaaaacgaaagctgcctggcgacccgcgaaaccagcagcaccacccgcggcagctgcctgccgccgcagaaaaccagcctgatgatgaccctgtgcctgggcagcatttatgaagatctgaaaatgtatcagaccgaatttcaggcgattaacgcggcgctgcagaaccataaccatcagcagattattctggataaaggcatgctggtggcgattgatgaactgatgcagagcctgaaccataacggcgaaaccctgcgccagaaaccgccggtgggcgaagcggatccgtatcgcgtgaaaatgaaactgtgcattctgctgcatgcgtttagcacccgcgtggtgaccattaaccgcgtgatgggctatctgagcagc

SEQ ID NO: 49 - DNA, 939 bp, synthetic construct
  source 1..939: mol_type = other DNA
ccgtgggaactggaaaaagatgtgtatgtggtggaagtggattggaccccggatgcgccgggcgaaaccgtgaacctgacctgcgataccccggaagaagatgatattacctggaccagcgatcagcgccatggcgtgattggcagcggcaaaaccctgaccattaccgtgaaagaatttctggatgcgggccagtatacctgccataaaggcggcgaaaccctgagccatagccatctgctgctgcataaaaaagaaaacggcatttggagcaccgaaattctgaaaaactttaaaaacaaaacctttctgaaatgcgaagcgccgaactatagcggccgctttacctgcagctggctggtgcagcgcaacatggatctgaaatttaacattaaaagcagcagcagcagcccggatagccgcgcggtgacctgcggcatggcgagcctgagcgcggaaaaagtgaccctggatcagcgcgattatgaaaaatatagcgtgagctgccaggaagatgtgacctgcccgaccgcggaagaaaccctgccgattgaactggcgctggaagcgcgccagcagaacaaatatgaaaactatagcaccagcttttttattcgcgatattattaaaccggatccgccgaaaaacctgcagatgaaaccgctgaaaaacagccaggtggaagtgagctgggaatatccggatagctggagcaccccgcatagctattttagcctgaaattttttgtgcgcattcagcgcaaaaaagaaaaaatgaaagaaaccgaagaaggctgcaaccagaaaggcgcgtttctggtggaaaaaaccagcaccgaagtgcagtgcaaaggcggcaacgtgtgcgtgcaggcgcaggatcgctattataacagcagctgcagcaaatgggcgtgcgtgccgtgccgcgtgcgcagc

SEQ ID NO: 50 - DNA, 939 bp, synthetic construct
  source 1..939: mol_type = other DNA
cagtgggaactggaaaaagatgtgtatgtggtggaagtggattggaccccggatgcgccgggcgaaaccgtgaacctgacctgcgataccccggaagaagatgatattacctggaccagcgatcagcgccatggcgtgattggcagcggcaaaaccctgaccattaccgtgaaagaatttctggatgcgggccagtatacctgccataaaggcggcgaaaccctgagccatagccatctgctgctgcataaaaaagaaaacggcatttggagcaccgaaattctgaaaaactttaaaaacaaaacctttctgaaatgcgaagcgccgaactatagcggccgctttacctgcagctggctggtgcagcgcaacatggatctgaaatttaacattaaaagcagcagcagcagcccggatagccgcgcggtgacctgcggcatggcgagcctgagcgcggaaaaagtgaccctggatcagcgcgattatgaaaaatatagcgtgagctgccaggaagatgtgacctgcccgaccgcggaagaaaccctgccgattgaactggcgctggaagcgcgccagcagaacaaatatgaaaactatagcaccagcttttttattcgcgatattattaaaccggatccgccgaaaaacctgcagatgaaaccgctgaaaaacagccaggtggaagtgagctgggaatatccggatagctggagcaccccgcatagctattttagcctgaaattttttgtgcgcattcagcgcaaaaaagaaaaaatgaaagaaaccgaagaaggctgcaaccagaaaggcgcgtttctggtggaaaaaaccagcaccgaagtgcagtgcaaaggcggcaacgtgtgcgtgcaggcgcaggatcgctattataacagcagctgcagcaaatgggcgtgcgtgccgtgccgcgtgcgcagc

SEQ ID NO: 51 - DNA, 939 bp, synthetic construct
  source 1..939: mol_type = other DNA
aactgggaactggaaaaagatgtgtatgtggtggaagtggattggaccccggatgcgccgggcgaaaccgtgaacctgacctgcgataccccggaagaagatgatattacctggaccagcgatcagcgccatggcgtgattggcagcggcaaaaccctgaccattaccgtgaaagaatttctggatgcgggccagtatacctgccataaaggcggcgaaaccctgagccatagccatctgctgctgcataaaaaagaaaacggcatttggagcaccgaaattctgaaaaactttaaaaacaaaacctttctgaaatgcgaagcgccgaactatagcggccgctttacctgcagctggctggtgcagcgcaacatggatctgaaatttaacattaaaagcagcagcagcagcccggatagccgcgcggtgacctgcggcatggcgagcctgagcgcggaaaaagtgaccctggatcagcgcgattatgaaaaatatagcgtgagctgccaggaagatgtgacctgcccgaccgcggaagaaaccctgccgattgaactggcgctggaagcgcgccagcagaacaaatatgaaaactatagcaccagcttttttattcgcgatattattaaaccggatccgccgaaaaacctgcagatgaaaccgctgaaaaacagccaggtggaagtgagctgggaatatccggatagctggagcaccccgcatagctattttagcctgaaattttttgtgcgcattcagcgcaaaaaagaaaaaatgaaagaaaccgaagaaggctgcaaccagaaaggcgcgtttctggtggaaaaaaccagcaccgaagtgcagtgcaaaggcggcaacgtgtgcgtgcaggcgcaggatcgctattataacagcagctgcagcaaatgggcgtgcgtgccgtgccgcgtgcgcagc

SEQ ID NO: 52 - DNA, 276 bp, Homo sapiens
  source 1..276: mol_type = genomic DNA
gcgccggatgtgcaggattgcccggaatgcaccctgcaggaaaacccgttttttagccagccgggcgcgccgattctgcagtgcatgggctgctgctttagccgcgcgtatccgaccccgctgcgcagcaaaaaaaccatgctggtgcagaaaaacgtgaccagcgaaagcacctgctgcgtggcgaaaagctataaccgcgtgaccgtgatgggcggctttaaagtggaaaaccataccgcgtgccattgcagcacctgctattatcataaaagc

SEQ ID NO: 53 - DNA, 363 bp, Homo sapiens
  source 1..363: mol_type = genomic DNA
agccgcgaaccgctgcgcccgtggtgccatccgattaacgcgattctggcggtggaaaaagaaggctgcccggtgtgcattaccgtgaacaccaccatttgcgcgggctattgcccgaccatgatgcgcgtgctgcaggcggtgctgccgccgctgccgcaggtggtgtgcacctatcgcgatgtgcgctttgaaagcattcgcctgccgggctgcccgcgcggcgtggatccggtggtgagctttccggtggcgctgagctgccgctgcggcccgtgccgccgcagcaccagcgattgcggcggcccgaaagatcatccgctgacctgcgatcatccgcagctgagcggcctgctgtttctg

SEQ ID NO: 54 - DNA, 354 bp, Homo sapiens
  source 1..354: mol_type = genomic DNA
ttttgcattccgaccgaatataccatgcatattgaacgccgcgaatgcgcgtattgcctgaccattaacaccaccatttgcgcgggctattgcatgacccgcgatattaacggcaaactgtttctgccgaaatatgcgctgagccaggatgtgtgcacctatcgcgattttatttatcgcaccgtggaaattccgggctgcccgctgcatgtggcgccgtattttagctatccggtggcgctgagctgcaaatgcggcaaatgcaacaccgattatagcgattgcattcatgaagcgattaaaaccaactattgcaccaaaccgcagaaaagctatctggtgggctttagcgtg

SEQ ID NO: 55 - DNA, 333 bp, Homo sapiens
  source 1..333: mol_type = genomic DNA
aacagctgcgaactgaccaacattaccattgcgattgaaaaagaagaatgccgcttttgcattagcattaacaccacctggtgcgcgggctattgctatacccgcgatctggtgtataaagatccggcgcgcccgaaaattcagaaaacctgcacctttaaagaactggtgtatgaaaccgtgcgcgtgccgggctgcgcgcatcatgcggatagcctgtatacctatccggtggcgacccagtgccattgcggcaaatgcgatagcgatagcaccgattgcaccgtgcgcggcctgggcccgagctattgcagctttggcgaaatgaaagaa

SEQ ID NO: 56 - DNA, 435 bp, Homo sapiens
  source 1..435: mol_type = genomic DNA
agcaaagaaccgctgcgcccgcgctgccgcccgattaacgcgaccctggcggtggaaaaagaaggctgcccggtgtgcattaccgtgaacaccaccatttgcgcgggctattgcccgaccatgacccgcgtgctgcagggcgtgctgccggcgctgccgcaggtggtgtgcaactatcgcgatgtgcgctttgaaagcattcgcctgccgggctgcccgcgcggcgtgaacccggtggtgagctatgcggtggcgctgagctgccagtgcgcgctgtgccgccgcagcaccaccgattgcggcggcccgaaagatcatccgctgacctgcgatgatccgcgctttcaggcgagcagcagcagcaaagcgccgccgccgagcctgccgagcccgagccgcctgccgggcccgagcgataccccgattctgccgcag

SEQ ID NO: 57 - DNA, 411 bp, Homo sapiens
  source 1..411: mol_type = genomic DNA
agcaaagaaccgctgcgcccgcgctgccgcccgattaacgcgaccctggcggtggaaaaagaaggctgcccggtgtgcattaccgtgaacaccaccatttgcgcgggctattgcccgaccatgacccgcgtgctgcagggcgtgctgccggcgctgccgcaggtggtgtgcaactatcgcgatgtgcgctttgaaagcattcgcctgccgggctgcccgcgcggcgtgaacccggtggtgagctatgcggtggcgctgagctgccagtgcgcgctgtgccgccgcagcaccaccgattgcggcggcccgaaagatcatccgctgacctgcgatgatccgcgctttcaggatagcagcagcagcaaagcgccgccgccgagcctgccgagcccgagccgcctgccgggcccg

SEQ ID NO: 58 - DNA, 435 bp, Homo sapiens
  source 1..435: mol_type = genomic DNA
agcaaagaaccgctgcgcccgcgctgccgcccgattaacgcgaccctggcggtggaaaaagaaggctgcccggtgtgcattaccgtgaacaccaccatttgcgcgggctattgcccgaccatgacccgcgtgctgcagggcgtgctgccggcgctgccgcaggtggtgtgcaactatcgcgatgtgcgctttgaaagcattcgcctgccgggctgcccgcgcggcgtgaacccggtggtgagctatgcggtggcgctgagctgccagtgcgcgctgtgccgccgcagcaccaccgattgcggcggcccgaaagatcatccgctgacctgcgatgatccgcgctttcaggatagcagcagcagcaaagcgccgccgccgagcctgccgagcccgagccgcctgccgggcccgagcgataccccgattctgccgcag

SEQ ID NO: 59 - DNA, 435 bp, Homo sapiens
  source 1..435: mol_type = genomic DNA
agccgcgaaatgctgcgcccgcgctgccgcccgattaacgcgaccctggcggtggaaaaagaaggctgcccggtgtgcattaccgtgaacaccaccatttgcgcgggctattgcccgaccatgacccgcgtgctgcagggcgtgctgccggcgctgccgcaggtggtgtgcaactatcgcgatgtgcgctttgaaagcattcgcctgccgggctgcccgcgcggcgtgaacccggtggtgagctatgcggtggcgctgagctgccagtgcgcgctgtgccgccgcagcaccaccgattgcggcggcccgaaagatcatccgctgacctgcgatgatccgcgctttcaggcgagcagcagcagcaaagcgccgccgccgagcctgccgagcccgagccgcctgccgggcccgagcgataccccgattctgccgcag

SEQ ID NO: 60 - DNA, 435 bp, Homo sapiens; identical to SEQ ID NO: 59
  source 1..435: mol_type = genomic DNA

SEQ ID NO: 61 - DNA, 276 bp, synthetic construct
  source 1..276: mol_type = other DNA
ccgccggatgtgcaggattgcccggaatgcaccctgcaggaaaacccgttttttagccagccgggcgcgccgattctgcagtgcatgggctgctgctttagccgcgcgtatccgaccccgctgcgcagcaaaaaaaccatgctggtgcagaaaaacgtgaccagcgaaagcacctgctgcgtggcgaaaagctataaccgcgtgaccgtgatgggcggctttaaagtggaaaaccataccgcgtgccattgcagcacctgctattatcataaaagc

SEQ ID NO: 62 - DNA, 276 bp, synthetic construct
  source 1..276: mol_type = other DNA
cagccggatgtgcaggattgcccggaatgcaccctgcaggaaaacccgttttttagccagccgggcgcgccgattctgcagtgcatgggctgctgctttagccgcgcgtatccgaccccgctgcgcagcaaaaaaaccatgctggtgcagaaaaacgtgaccagcgaaagcacctgctgcgtggcgaaaagctataaccgcgtgaccgtgatgggcggctttaaagtggaaaaccataccgcgtgccattgcagcacctgctattatcataaaagc

SEQ ID NO: 63 - DNA, 276 bp, synthetic construct
  source 1..276: mol_type = other DNA
aacccggatgtgcaggattgcccggaatgcaccctgcaggaaaacccgttttttagccagccgggcgcgccgattctgcagtgcatgggctgctgctttagccgcgcgtatccgaccccgctgcgcagcaaaaaaaccatgctggtgcagaaaaacgtgaccagcgaaagcacctgctgcgtggcgaaaagctataaccgcgtgaccgtgatgggcggctttaaagtggaaaaccataccgcgtgccattgcagcacctgctattatcataaaagc

SEQ ID NO: 64 - DNA, 288 bp, Mus musculus
  source 1..288: mol_type = genomic DNA
ctgccggatggcgattttattattcagggctgcccggaatgcaaactgaaagaaaacaaatattttagcaaactgggcgcgccgatttatcagtgcatgggctgctgctttagccgcgcgtatccgaccccggcgcgcagcaaaaaaaccatgctggtgccgaaaaacattaccagcgaagcgacctgctgcgtggcgaaagcgtttaccaaagcgaccgtgatgggcaacgcgcgcgtggaaaaccataccgaatgccattgcagcacctgctattatcataaaagc

SEQ ID NO: 65 - DNA, 363 bp, Mus musculus
  source 1..363: mol_type = genomic DNA
agccgcggcccgctgcgcccgctgtgccgcccggtgaacgcgaccctggcggcggaaaacgaattttgcccggtgtgcattacctttaccaccagcatttgcgcgggctattgcccgagcatggtgcgcgtgctgccggcggcgctgccgccggtgccgcagccggtgtgcacctatcgcgaactggcgtttgcgagcgtgcgcctgccgggctgcccgccgggcgtggatccgattgtgagctttccggtggcgctgagctgccgctgcggcccgtgccgcctgagcagcagcgattgcggcggcccgcgcacccagccgatggcgtgcgatctgccgcatctgccgggcctgctgctgctg

SEQ ID NO: 66 - DNA, 354 bp, Mus musculus
  source 1..354: mol_type = genomic DNA
ttttgcattccgaccgaatataccatgtatgtggatcgccgcgaatgcgcgtattgcctgaccattaacaccaccatttgcgcgggctattgcatgacccgcgatattaacggcaaactgtttctgccgaaatatgcgctgagccaggatgtgtgcacctatcgcgattttatttatcgcaccgtggaaattccgggctgcccgcatcatgtgaccccgtattttagctttccggtggcggtgagctgcaaatgcggcaaatgcaacaccgataacagcgattgcattcatgaagcggtgcgcaccaactattgcaccaaaccgcagagcttttatctgggcggctttagcgtg

SEQ ID NO: 67 - DNA, 327 bp, Mus musculus
  source 1..327: mol_type = genomic DNA
tgcgaactgaccaacattaccattagcgtggaaaaagaagaatgccgcttttgcattagcattaacaccacctggtgcgcgggctattgctatacccgcgatctggtgtataaagatccggcgcgcccgaacacccagaaagtgtgcacctttaaagaactggtgtatgaaaccgtgcgcctgccgggctgcgcgcgccatagcgatagcctgtatacctatccggtggcgaccgaatgccattgcggcaaatgcgatagcgatagcaccgattgcaccgtgcgcggcctgggcccgagctattgcagctttagcgaaatgaaagaa

SEQ ID NO: 68 - DNA, 288 bp, synthetic construct
  source 1..288: mol_type = other DNA
ccgccggatggcgattttattattcagggctgcccggaatgcaaactgaaagaaaacaaatattttagcaaactgggcgcgccgatttatcagtgcatgggctgctgctttagccgcgcgtatccgaccccggcgcgcagcaaaaaaaccatgctggtgccgaaaaacattaccagcgaagcgacctgctgcgtggcgaaagcgtttaccaaagcgaccgtgatgggcaacgcgcgcgtggaaaaccataccgaatgccattgcagcacctgctattatcataaaagc

SEQ ID NO: 69 - DNA, 288 bp, synthetic construct
  source 1..288: mol_type = other DNA
cagccggatggcgattttattattcagggctgcccggaatgcaaactgaaagaaaacaaatattttagcaaactgggcgcgccgatttatcagtgcatgggctgctgctttagccgcgcgtatccgaccccggcgcgcagcaaaaaaaccatgctggtgccgaaaaacattaccagcgaagcgacctgctgcgtggcgaaagcgtttaccaaagcgaccgtgatgggcaacgcgcgcgtggaaaaccataccgaatgccattgcagcacctgctattatcataaaagc

SEQ ID NO: 70 - DNA, 288 bp, synthetic construct
  source 1..288: mol_type = other DNA
aacccggatggcgattttattattcagggctgcccggaatgcaaactgaaagaaaacaaatattttagcaaactgggcgcgccgatttatcagtgcatgggctgctgctttagccgcgcgtatccgaccccggcgcgcagcaaaaaaaccatgctggtgccgaaaaacattaccagcgaagcgacctgctgcgtggcgaaagcgtttaccaaagcgaccgtgatgggcaacgcgcgcgtggaaaaccataccgaatgccattgcagcacctgctattatcataaaagc